European Patent Application EP 4 461 739 A2, published November 13, 2024. Title: BICYCLIC PEPTIDE LIGANDS SPECIFIC FOR NECTIN-4. Applicant: BicycleTx Limited. The sequence listing filed with the application follows.

SEQUENCE LISTING (5 sequences)

SEQ ID NO: 1 - protein, 15 aa, synthetic construct
  REGION 1..15: note = synthetic
  SITE 3: note = 1- Naphthylalanine
  SITE 4: note = D-aspartic acid
  SITE 7: note = HomoArginine
  SITE 13: note = Hydroxyproline
CPXXCMXDWSTPXWC

SEQ ID NO: 2 - protein, 24 aa, synthetic construct
  REGION 1..18: note = synthetic
  SITE 18..23: note = Sarcosine
  SITE 24: note = Fluorescein (Fl) labelled lysine
ACPFGCHTDWSWPIWCAXXXXXXK

SEQ ID NO: 3 - protein, 26 aa, synthetic construct
  SITE 1: note = Beta-alanine
  SITE 2..11: note = Sarcosine
  SITE 14: note = 1-Naphthylalanine
  SITE 15: note = D-aspartic acid
  SITE 18: note = HomoArginine
  SITE 24: note = Hydroxyproline
AXXXXXXXXXXCPXXCMXDWSTPXWC

SEQ ID NO: 4 - protein, 21 aa, synthetic construct
  SITE 1: note = Beta-alanine
  SITE 2..6: note = Sarcosine
  SITE 9: note = 1-Naphthylalanine
  SITE 10: note = D-aspartic acid
  SITE 13: note = HomoArginine
  SITE 19: note = Hydroxyproline
AXXXXXCPXXCMXDWSTPXWC

SEQ ID NO: 5 - protein, 27 aa, synthetic construct
  SITE 1: note = Beta-alanine
  SITE 2..11: note = Sarcosine
  SITE 15: note = 1-Naphthylalanine
  SITE 16: note = D-aspartic acid
  SITE 19: note = HomoArginine
  SITE 25: note = Hydroxyproline
AXXXXXXXXXXACPXXCMXDWSTPXWC